European Patent Application EP 4 269 607 A2, published November 1, 2023. Title: DETECTION OF TARGET NUCLEIC ACID SEQUENCES USING DIFFERENT DETECTION TEMPERATURES. Applicant: SEEGENE, INC. The sequence listing filed with the application follows.

SEQUENCE LISTING (18 sequences)

SEQ ID NO: 1 - DNA, 37 bp, synthetic construct
  misc_feature 1..37: note = NG-F
  misc_feature 22..26: note = n denotes deoxyinosine
  source 1..37: mol_type = other DNA
tacgcctgctactttcacgctnnnnngtaatcagatg

SEQ ID NO: 2 - DNA, 37 bp, synthetic construct
  misc_feature 1..37: note = NG-R
  misc_feature 22..26: note = n denotes deoxyinosine
  source 1..37: mol_type = other DNA
caatggatcggtatcactcgcnnnnncgagcaagaac

SEQ ID NO: 3 - DNA, 34 bp, synthetic construct
  misc_feature 1..34: note = NG-PTO
  source 1..34: mol_type = other DNA
gtacgcgatacgggcccctcattggcgtgtttcg

SEQ ID NO: 4 - DNA, 39 bp, synthetic construct
  misc_feature 1..39: note = NG-CTO
  source 1..39: mol_type = other DNA
tttttttttttttttttttgtactgcccgtatcgcgtac

SEQ ID NO: 5 - DNA, 40 bp, synthetic construct
  misc_feature 1..40: note = CT-F
  misc_feature 26..30: note = n denotes deoxyinosine
  source 1..40: mol_type = other DNA
gagttttaaaatgggaaattctggtnnnnntttgtataac

SEQ ID NO: 6 - DNA, 40 bp, synthetic construct
  misc_feature 1..40: note = CT-R
  misc_feature 26..30: note = n denotes deoxyinosine
  source 1..40: mol_type = other DNA
ccaattgtaatagaagcattggttgnnnnnttattggaga

SEQ ID NO: 7 - DNA, 39 bp, synthetic construct
  misc_feature 1..39: note = CT-PTO
  source 1..39: mol_type = other DNA
gattacgcgaccgcatcagaagctgtcattttggctgcg

SEQ ID NO: 8 - DNA, 39 bp, synthetic construct
  misc_feature 1..39: note = CT-CTO
  source 1..39: mol_type = other DNA
gcgctggataccctggacgatatgtgcggtcgcgtaatc

SEQ ID NO: 9 - DNA, 26 bp, synthetic construct
  misc_feature 1..26: note = CT-P
  source 1..26: mol_type = other DNA
catcagaagctgtcattttggctgcg

SEQ ID NO: 10 - DNA, 32 bp, synthetic construct
  misc_feature 1..32: note = M677-F
  misc_feature 18..22: note = n denotes deoxyinosine
  source 1..32: mol_type = other DNA
ccaccccgaagcagggannnnngaggctgacc

SEQ ID NO: 11 - DNA, 34 bp, synthetic construct
  misc_feature 1..34: note = M677-R
  misc_feature 20..24: note = n denotes deoxyinosine
  source 1..34: mol_type = other DNA
caagtgatgcccatgtcggnnnnngccttcacaa

SEQ ID NO: 12 - DNA, 37 bp, synthetic construct
  misc_feature 1..37: note = M677-W-PTO
  source 1..37: mol_type = other DNA
ggtcccgacgttagctcccgcagacaccttctccttc

SEQ ID NO: 13 - DNA, 39 bp, synthetic construct
  misc_feature 1..39: note = M677-W-CTO
  source 1..39: mol_type = other DNA
cctcggtgccacgccatcggttcttctaacgtcgggacc

SEQ ID NO: 14 - DNA, 38 bp, synthetic construct
  misc_feature 1..38: note = M677-M-PTO
  source 1..38: mol_type = other DNA
acgtcgattcgcactcccgcagacaccttctccttcaa

SEQ ID NO: 15 - DNA, 38 bp, synthetic construct
  misc_feature 1..38: note = M677-M-CTO
  source 1..38: mol_type = other DNA
tttttttttttttttttttttattctgcgaatcgacgt

SEQ ID NO: 16 - DNA, 38 bp, synthetic construct
  misc_feature 1..38: note = MG-F
  misc_feature 23..27: note = n denotes deoxyinosine
  source 1..38: mol_type = other DNA
aaaacccacggaaatgatgagannnnnattggttctac

SEQ ID NO: 17 - DNA, 41 bp, synthetic construct
  misc_feature 1..41: note = MG-R
  misc_feature 27..30: note = n denotes deoxyinosine
  source 1..41: mol_type = other DNA
ctcgttaatttacctattccattttgnnnnnctgataaaag

SEQ ID NO: 18 - DNA, 28 bp, synthetic construct
  misc_feature 1..28: note = MG-P
  source 1..28: mol_type = other DNA
gagttctttcaagaacagcaagaggtgt